European Patent Application EP 4 549 555 A2, published May 7, 2025. Title: CCR4 TARGETED CHIMERIC ANTIGEN RECEPTOR MODIFIED T CELLS FOR TREATMENT OF CCR4 POSITIVE MALIGNANCIES. Applicant: City of Hope. Application EP. The sequence listing filed with the application follows.

SEQUENCE LISTING (48 sequences)

SEQ ID NO: 1 - protein, 246 aa, synthetic construct
  REGION 1..246: note = huCCR4 scFv
QVQLVQSGAEVVKPGASVKISCKASGYTFTDHAIHWVKQNPGQRLEWIGYFSPGNDDFKYNERFKGKATLTADTSASTAYVELSSLRSEDTAVYFCTRSLNMAYWGQGTLVTVSSGSTSGGGSGGGSGGGGSSDIVMSQSPDSLAVSLGERVTLNCKSSQSLLYSGNQKNYLAWYQQKPGQSPKLLIYWASARESGVPDRFSGSGSGTDFTLTISSVQAEDVAVYYCQQYYSYPLTFGAGTKLELK

SEQ ID NO: 2 - protein, 10 aa, synthetic construct
  REGION 1..10: note = linker
GGGSSGGGSG

SEQ ID NO: 3 - protein, 12 aa, synthetic construct
  REGION 1..12: note = IgG4 hinge (S228P)
ESKYGPPCPPCP

SEQ ID NO: 4 - protein, 12 aa, synthetic construct
  REGION 1..12: note = IgG4 hinge
ESKYGPPCPSCP

SEQ ID NO: 5 - protein, 22 aa, synthetic construct
  REGION 1..22: note = IgG4 hinge (S228P)+ linker
ESKYGPPCPPCPGGGSSGGGSG

SEQ ID NO: 6 - protein, 39 aa, synthetic construct
  REGION 1..39: note = CD28 hinge
IEVMYPPPYLDNEKSNGTIIHVKGKHLCPSPLFPGPSKP

SEQ ID NO: 7 - protein, 48 aa, synthetic construct
  REGION 1..48: note = CD8 hinge-48aa
AKPTTTPAPRPPTPAPTIASQPLSLRPEACRPAAGGAVHTRGLDFACD

SEQ ID NO: 8 - protein, 45 aa, synthetic construct
  REGION 1..45: note = CD8 hinge-45aa
TTTPAPRPPTPAPTIASQPLSLRPEACRPAAGGAVHTRGLDFACD

SEQ ID NO: 9 - protein, 129 aa, synthetic construct
  REGION 1..129: note = IgG4(HL-CH3) (S228P)
ESKYGPPCPPCPGGGSSGGGSGGQPREPQVYTLPPSQEEMTKNQVSLTCLVKGFYPSDIAVEWESNGQPENNYKTTPPVLDSDGSFFLYSRLTVDKSRWQEGNVFSCSVMHEALHNHYTQKSLSLSLGK

SEQ ID NO: 10 - protein, 229 aa, synthetic construct
  REGION 1..229: note = IgG4(L235E,N297Q)
ESKYGPPCPSCPAPEFEGGPSVFLFPPKPKDTLMISRTPEVTCVVVDVSQEDPEVQFNWYVDGVEVHQAKTKPREEQFQSTYRVVSVLTVLHQDWLNGKEYKCKVSNKGLPSSIEKTISKAKGQPREPQVYTLPPSQEEMTKNQVSLTCLVKGFYPSDIAVEWESNGQPENNYKTTPPVLDSDGSFFLYSRLTVDKSRWQEGNVFSCSVMHEALHNHYTQKSLSLSLGK

SEQ ID NO: 11 - protein, 229 aa, synthetic construct
  REGION 1..229: note = IgG4(S228P, L235E,N297Q)
ESKYGPPCPPCPAPEFEGGPSVFLFPPKPKDTLMISRTPEVTCVVVDVSQEDPEVQFNWYVDGVEVHQAKTKPREEQFQSTYRVVSVLTVLHQDWLNGKEYKCKVSNKGLPSSIEKTISKAKGQPREPQVYTLPPSQEEMTKNQVSLTCLVKGFYPSDIAVEWESNGQPENNYKTTPPVLDSDGSFFLYSRLTVDKSRWQEGNVFSCSVMHEALHNHYTQKSLSLSLGK

SEQ ID NO: 12 - protein, 107 aa, synthetic construct
  REGION 1..107: note = IgG4(CH3)
GQPREPQVYTLPPSQEEMTKNQVSLTCLVKGFYPSDIAVEWESNGQPENNYKTTPPVLDSDGSFFLYSRLTVDKSRWQEGNVFSCSVMHEALHNHYTQKSLSLSLGK

SEQ ID NO: 13 - protein, 21 aa, synthetic construct
  REGION 1..21: note = CD3z
LCYLLDGILFIYGVILTALFL

SEQ ID NO: 14 - protein, 27 aa, synthetic construct
  REGION 1..27: note = CD28
FWVLVVVGGVLACYSLLVTVAFIIFWV

SEQ ID NO: 15 - protein, 28 aa, synthetic construct
  REGION 1..28: note = CD28(M)
MFWVLVVVGGVLACYSLLVTVAFIIFWV

SEQ ID NO: 16 - protein, 22 aa, synthetic construct
  REGION 1..22: note = CD4
MALIVLGGVAGLLLFIGLGIFF

SEQ ID NO: 17 - protein, 21 aa, synthetic construct
  REGION 1..21: note = CD8tm
IYIWAPLAGTCGVLLLSLVIT

SEQ ID NO: 18 - protein, 23 aa, synthetic construct
  REGION 1..23: note = CD8tm2
IYIWAPLAGTCGVLLLSLVITLY

SEQ ID NO: 19 - protein, 24 aa, synthetic construct
  REGION 1..24: note = CD8tm3
IYIWAPLAGTCGVLLLSLVITLYC

SEQ ID NO: 20 - protein, 27 aa, synthetic construct
  REGION 1..27: note = 41BB
IISFFLALTSTALLFLLFFLTLRFSVV

SEQ ID NO: 21 - protein, 112 aa, synthetic construct
  REGION 1..112: note = CD3 Zeta
RVKFSRSADAPAYQQGQNQLYNELNLGRREEYDVLDKRRGRDPEMGGKPRRKNPQEGLYNELQKDKMAEAYSEIGMKGERRRGKGHDGLYQGLSTATKDTYDALHMQALPPR

SEQ ID NO: 22 - protein, 41 aa, synthetic construct
  REGION 1..41: note = CD28
RSKRSRLLHSDYMNMTPRRPGPTRKHYQPYAPPRDFAAYRS

SEQ ID NO: 23 - protein, 41 aa, synthetic construct
  REGION 1..41: note = CD28gg
RSKRSRGGHSDYMNMTPRRPGPTRKHYQPYAPPRDFAAYRS

SEQ ID NO: 24 - protein, 42 aa, synthetic construct
  REGION 1..42: note = 41BB
KRGRKKLLYIFKQPFMRPVQTTQEEDGCSCRFPEEEEGGCEL

SEQ ID NO: 25 - protein, 42 aa, synthetic construct
  REGION 1..42: note = OX40
ALYLLRRDQRLPPDAHKPPGGGSFRTPIQEEQADAHSTLAKI

SEQ ID NO: 26 - protein, 323 aa, synthetic construct
  REGION 1..323: note = truncated CD19R
MPPPRLLFFLLFLTPMEVRPEEPLVVKVEEGDNAVLQCLKGTSDGPTQQLTWSRESPLKPFLKLSLGLPGLGIHMRPLAIWLFIFNVSQQMGGFYLCQPGPPSEKAWQPGWTVNVEGSGELFRWNVSDLGGLGCGLKNRSSEGPSSPSGKLMSPKLYVWAKDRPEIWEGEPPCVPPRDSLNQSLSQDLTMAPGSTLWLSCGVPPDSVSRGPLSWTHVHPKGPKSLLSLELKDDRPARDMWVMETGLLLPRATAQDAGKYYCHRGNLTMSFHLEITARPVLWHWLLRTGGWKVSAVTLAYLIFCLCSLVGILHLQRALVLRRKR

SEQ ID NO: 27 - protein, 24 aa, synthetic construct
  REGION 1..24: note = ribosomal skip sequence
LEGGGEGRGSLLTCGDVEENPGPR

SEQ ID NO: 28 - protein, 354 aa, synthetic construct
  REGION 1..354: note = truncated EGFR
LVTSLLLCELPHPAFLLIPRKVCNGIGIGEFKDSLSINATNIKHFKNCTSISGDLHILPVAFRGDSFTHTPPLDPQELDILKTVKEITGFLLIQAWPENRTDLHAFENLEIIRGRTKQHGQFSLAVVSLNITSLGLRSLKEISDGDVIISGNKNLCYANTINWKKLFGTSGQKTKIISNRGENSCKATGQVCHALCSPEGCWGPEPRDCVSCRNVSRGRECVDKCNLLEGEPREFVENSECIQCHPECLPQAMNITCTGRGPDNCIQCAHYIDGPHCVKTCPAGVMGENNTLVWKYADAGHVCHLCHPNCTYGCTGPGLEGCPTNGPKIPSIATGMVGALLLLLVVALGIGLFM

SEQ ID NO: 29 - protein, 456 aa, synthetic construct
  REGION 1..456: note = CCR4scFv-Linker-CD4tm-41BB-Zeta with GMCSFRa signal sequence
MLLLVTSLLLCELPHPAFLLIPQVQLVQSGAEVKKPGASVKVSCKASGYTFASYYMHWMRQAPGQGLEWIGWINPGNVNTKYNEKFKGRATLTVDTSTNTAYMELSSLRSEDTAVYYCARSTYYRPLDYWGQGTLVTVSSSGGGSGGGGSGGGGSDIVMTQSPDSLAVSLGERATINCKSSQSILYSSNQKNYLAWYQQKPGQSPKLLIYWASTRESGVPDRFSGSGSGTDFTLTISSLQAEDVAVYYCHQYLSSYTFGQGTKLEIKGGGSSGGGSGMALIVLGGVAGLLLFIGLGIFFKRGRKKLLYIFKQPFMRPVQTTQEEDGCSCRFPEEEEGGCELGGGRVKFSRSADAPAYQQGQNQLYNELNLGRREEYDVLDKRRGRDPEMGGKPRRKNPQEGLYNELQKDKMAEAYSEIGMKGERRRGKGHDGLYQGLSTATKDTYDALHMQALPPR

SEQ ID NO: 30 - protein, 675 aa, synthetic construct
  REGION 1..675: note = CCR4scFv-IgG4(L235E,N297Q)-CD4tm-41BB-Zeta with GMCSFRa signal sequence
MLLLVTSLLLCELPHPAFLLIPQVQLVQSGAEVKKPGASVKVSCKASGYTFASYYMHWMRQAPGQGLEWIGWINPGNVNTKYNEKFKGRATLTVDTSTNTAYMELSSLRSEDTAVYYCARSTYYRPLDYWGQGTLVTVSSSGGGSGGGGSGGGGSDIVMTQSPDSLAVSLGERATINCKSSQSILYSSNQKNYLAWYQQKPGQSPKLLIYWASTRESGVPDRFSGSGSGTDFTLTISSLQAEDVAVYYCHQYLSSYTFGQGTKLEIKESKYGPPCPPCPAPEFEGGPSVFLFPPKPKDTLMISRTPEVTCVVVDVSQEDPEVQFNWYVDGVEVHNAKTKPREEQFQSTYRVVSVLTVLHQDWLNGKEYKCKVSNKGLPSSIEKTISKAKGQPREPQVYTLPPSQEEMTKNQVSLTCLVKGFYPSDIAVEWESNGQPENNYKTTPPVLDSDGSFFLYSRLTVDKSRWQEGNVFSCSVMHEALHNHYTQKSLSLSLGKMALIVLGGVAGLLLFIGLGIFFKRGRKKLLYIFKQPFMRPVQTTQEEDGCSCRFPEEEEGGCELGGGRVKFSRSADAPAYQQGQNQLYNELNLGRREEYDVLDKRRGRDPEMGGKPRRKNPQEGLYNELQKDKMAEAYSEIGMKGERRRGKGHDGLYQGLSTATKDTYDALHMQALPPR

SEQ ID NO: 31 - protein, 575 aa, synthetic construct
  REGION 1..575: note = CCR4scFv-IgG4(HL-CH3)-CD4tm-41BB-Zeta with GMCSFRa signal sequence
MLLLVTSLLLCELPHPAFLLIPQVQLVQSGAEVKKPGASVKVSCKASGYTFASYYMHWMRQAPGQGLEWIGWINPGNVNTKYNEKFKGRATLTVDTSTNTAYMELSSLRSEDTAVYYCARSTYYRPLDYWGQGTLVTVSSSGGGSGGGGSGGGGSDIVMTQSPDSLAVSLGERATINCKSSQSILYSSNQKNYLAWYQQKPGQSPKLLIYWASTRESGVPDRFSGSGSGTDFTLTISSLQAEDVAVYYCHQYLSSYTFGQGTKLEIKESKYGPPCPPCPGGGSSGGGSGGQPREPQVYTLPPSQEEMTKNQVSLTCLVKGFYPSDIAVEWESNGQPENNYKTTPPVLDSDGSFFLYSRLTVDKSRWQEGNVFSCSVMHEALHNHYTQKSLSLSLGKMALIVLGGVAGLLLFIGLGIFFKRGRKKLLYIFKQPFMRPVQTTQEEDGCSCRFPEEEEGGCELGGGRVKFSRSADAPAYQQGQNQLYNELNLGRREEYDVLDKRRGRDPEMGGKPRRKNPQEGLYNELQKDKMAEAYSEIGMKGERRRGKGHDGLYQGLSTATKDTYDALHMQALPPR

SEQ ID NO: 32 - protein, 118 aa, synthetic construct
  REGION 1..118: note = huCCR4 scFv V
QVQLVQSGAEVKKPGASVKVSCKASGYTFASYYMHWMRQAPGQGLEWIGWINPGNVNTKYNEKFKGRATLTVDTSTNTAYMELSSLRSEDTAVYYCARSTYYRPLDYWGQGTLVTVSS

SEQ ID NO: 33 - protein, 112 aa, synthetic construct
  REGION 1..112: note = huCCR4 scFv V
DIVMTQSPDSLAVSLGERATMSCKSSQSILYSSNQKNYLAWYQQKPGQSPKLLIYWASTRESGVPDRFSGSGSGTDFTLTISSLQAEDVAVYYCHQYLSSYTFGQGTKLEIK

SEQ ID NO: 34 - protein, 118 aa, synthetic construct
  REGION 1..118: note = huCCR4 scFv V
QVQLVQSGAEVKKPGASVKVSCKASGYTFASQWMHWMRQAPGQGLEWIGWINPGNVNTKYNEKFKGRATLTVDTSTNTAYMELSSLRSEDTAVYYCARSTWYRPLDYWGQGTLVTVSS

SEQ ID NO: 35 - protein, 112 aa, synthetic construct
  REGION 1..112: note = huCCR4 scFv V
DIVMTQSPDSLAVSLGERATMSCKSSQSILYSSNQKNYLAWYQQKPGQSPKLLIYWASTRESGVPDRFSGSGSGTDFTLTISSLQAEDVAVYYCHQYISSYTFGQGTKLEIK

SEQ ID NO: 36 - protein, 118 aa, synthetic construct
  REGION 1..118: note = huCCR4 scFv V
QVQLVQSGAEVKKPGASVKVSCKASGYTFASAWMHWMRQAPGQGLEWIGWINPGNVNTKYNEKFKGRATLTVDTSTNTAYMELSSLRSEDTAVYYCARSTYYRPLDYWGQGTLVTVSS

SEQ ID NO: 37 - protein, 112 aa, synthetic construct
  REGION 1..112: note = huCCR4 scFv V
DIVMTQSPDSLAVSLGERATMSCKSSQSILYSSNQKNYLAWYQQKPGQSPKLLIYWASTRESGVPDRFSGSGSGTDFTLTISSLQAEDVAVYYCHQYMSSYTFGQGTKLEIK

SEQ ID NO: 38 - protein, 434 aa, synthetic construct
  REGION 1..434: note = CCR4scFv-Linker-CD4tm-41BB-Zeta
QVQLVQSGAEVKKPGASVKVSCKASGYTFASYYMHWMRQAPGQGLEWIGWINPGNVNTKYNEKFKGRATLTVDTSTNTAYMELSSLRSEDTAVYYCARSTYYRPLDYWGQGTLVTVSSSGGGSGGGGSGGGGSDIVMTQSPDSLAVSLGERATINCKSSQSILYSSNQKNYLAWYQQKPGQSPKLLIYWASTRESGVPDRFSGSGSGTDFTLTISSLQAEDVAVYYCHQYLSSYTFGQGTKLEIKGGGSSGGGSGMALIVLGGVAGLLLFIGLGIFFKRGRKKLLYIFKQPFMRPVQTTQEEDGCSCRFPEEEEGGCELGGGRVKFSRSADAPAYQQGQNQLYNELNLGRREEYDVLDKRRGRDPEMGGKPRRKNPQEGLYNELQKDKMAEAYSEIGMKGERRRGKGHDGLYQGLSTATKDTYDALHMQALPPR

SEQ ID NO: 39 - protein, 653 aa, synthetic construct
  REGION 1..653: note = CCR4scFv-IgG4(L235E,N297Q)-CD4tm-41BB-Zeta
QVQLVQSGAEVKKPGASVKVSCKASGYTFASYYMHWMRQAPGQGLEWIGWINPGNVNTKYNEKFKGRATLTVDTSTNTAYMELSSLRSEDTAVYYCARSTYYRPLDYWGQGTLVTVSSSGGGSGGGGSGGGGSDIVMTQSPDSLAVSLGERATINCKSSQSILYSSNQKNYLAWYQQKPGQSPKLLIYWASTRESGVPDRFSGSGSGTDFTLTISSLQAEDVAVYYCHQYLSSYTFGQGTKLEIKESKYGPPCPPCPAPEFEGGPSVFLFPPKPKDTLMISRTPEVTCVVVDVSQEDPEVQFNWYVDGVEVHNAKTKPREEQFQSTYRVVSVLTVLHQDWLNGKEYKCKVSNKGLPSSIEKTISKAKGQPREPQVYTLPPSQEEMTKNQVSLTCLVKGFYPSDIAVEWESNGQPENNYKTTPPVLDSDGSFFLYSRLTVDKSRWQEGNVFSCSVMHEALHNHYTQKSLSLSLGKMALIVLGGVAGLLLFIGLGIFFKRGRKKLLYIFKQPFMRPVQTTQEEDGCSCRFPEEEEGGCELGGGRVKFSRSADAPAYQQGQNQLYNELNLGRREEYDVLDKRRGRDPEMGGKPRRKNPQEGLYNELQKDKMAEAYSEIGMKGERRRGKGHDGLYQGLSTATKDTYDALHMQALPPR

SEQ ID NO: 40 - protein, 553 aa, synthetic construct
  REGION 1..553: note = CCR4scFv-IgG4(HL-CH3)-CD4tm-41BB-Zeta
QVQLVQSGAEVKKPGASVKVSCKASGYTFASYYMHWMRQAPGQGLEWIGWINPGNVNTKYNEKFKGRATLTVDTSTNTAYMELSSLRSEDTAVYYCARSTYYRPLDYWGQGTLVTVSSSGGGSGGGGSGGGGSDIVMTQSPDSLAVSLGERATINCKSSQSILYSSNQKNYLAWYQQKPGQSPKLLIYWASTRESGVPDRFSGSGSGTDFTLTISSLQAEDVAVYYCHQYLSSYTFGQGTKLEIKESKYGPPCPPCPGGGSSGGGSGGQPREPQVYTLPPSQEEMTKNQVSLTCLVKGFYPSDIAVEWESNGQPENNYKTTPPVLDSDGSFFLYSRLTVDKSRWQEGNVFSCSVMHEALHNHYTQKSLSLSLGKMALIVLGGVAGLLLFIGLGIFFKRGRKKLLYIFKQPFMRPVQTTQEEDGCSCRFPEEEEGGCELGGGRVKFSRSADAPAYQQGQNQLYNELNLGRREEYDVLDKRRGRDPEMGGKPRRKNPQEGLYNELQKDKMAEAYSEIGMKGERRRGKGHDGLYQGLSTATKDTYDALHMQALPPR

SEQ ID NO: 41 - protein, 248 aa, synthetic construct
  REGION 1..248: note = tTA
MSRLDKSKVINSALELLNEVGIEGLTTRKLAQKLGVEQPTLYWHVKNKRALLDALAIEMLDRHHTHFCPLEGESWQDFLRNNAKSFRCALLSHRDGAKVHLGTRPTEKQYETLENQLAFLCQQGFSLENALYALSAVGHFTLGCVLEDQEHQVAKEERETPTTDSMPPLLRQAIELFDHQGAEPAFLFGLELIICGLEKQLKCESGGPADALDDFDLDMLPADALDDFDLDMLPADALDDLDLDMLPG

SEQ ID NO: 42 - protein, 595 aa, synthetic construct
  REGION 1..595: note = tTa-T2A-CD19t
MSRLDKSKVINSALELLNEVGIEGLTTRKLAQKLGVEQPTLYWHVKNKRALLDALAIEMLDRHHTHFCPLEGESWQDFLRNNAKSFRCALLSHRDGAKVHLGTRPTEKQYETLENQLAFLCQQGFSLENALYALSAVGHFTLGCVLEDQEHQVAKEERETPTTDSMPPLLRQAIELFDHQGAEPAFLFGLELIICGLEKQLKCESGGPADALDDFDLDMLPADALDDFDLDMLPADALDDLDLDMLPGLEGGGEGRGSLLTCGDVEENPGPRMPPPRLLFFLLFLTPMEVRPEEPLVVKVEEGDNAVLQCLKGTSDGPTQQLTWSRESPLKPFLKLSLGLPGLGIHMRPLAIWLFIFNVSQQMGGFYLCQPGPPSEKAWQPGWTVNVEGSGELFRWNVSDLGGLGCGLKNRSSEGPSSPSGKLMSPKLYVWAKDRPEIWEGEPPCVPPRDSLNQSLSQDLTMAPGSTLWLSCGVPPDSVSRGPLSWTHVHPKGPKSLLSLELKDDRPARDMWVMETGLLLPRATAQDAGKYYCHRGNLTMSFHLEITARPVLWHWLLRTGGWKVSAVTLAYLIFCLCSLVGILHLQRALVLRRKR

SEQ ID NO: 43 - protein, 245 aa, synthetic construct
  REGION 1..245: note = huCCR4 scFv
QVQLVQSGAEVKKPGASVKVSCKASGYTFASYYMHWMRQAPGQGLEWIGWINPGNVNTKYNEKFKGRATLTVDTSTNTAYMELSSLRSEDTAVYYCARSTYYRPLDYWGQGTLVTVSSSGGGSGGGGSGGGGSDIVMTQSPDSLAVSLGERATINCKSSQSILYSSNQKNYLAWYQQKPGQSPKLLIYWASTRESGVPDRFSGSGSGTDFTLTISSLQAEDVAVYYCHQYLSSYTFGQGTKLEIK

SEQ ID NO: 44 - protein, 236 aa, synthetic construct
  REGION 1..236: note = huCCR4 scFv
QVQLVQSGAEVKKPGASVKVSCKASGYTFASYYMHWMRQAPGQGLEWIGWINPGNVNTKYNEKFKGRATLTVDTSTNTAYMELSSLRSEDTAVYYCARSTYYRPLDYWGQGTLVTVSSSGGGGSDIVMTQSPDSLAVSLGERATINCKSSQSILYSSNQKNYLAWYQQKPGQSPKLLIYWASTRESGVPDRFSGSGSGTDFTLTISSLQAEDVAVYYCHQYLSSYTFGQGTKLEIK

SEQ ID NO: 45 - protein, 240 aa, synthetic construct
  REGION 1..240: note = huCCR4 scFv
QVQLVQSGAEVKKPGASVKVSCKASGYTFASYYMHWMRQAPGQGLEWIGWINPGNVNTKYNEKFKGRATLTVDTSTNTAYMELSSLRSEDTAVYYCARSTYYRPLDYWGQGTLVTVSSGGGGSGGGGSDIVMTQSPDSLAVSLGERATINCKSSQSILYSSNQKNYLAWYQQKPGQSPKLLIYWASTRESGVPDRFSGSGSGTDFTLTISSLQAEDVAVYYCHQYLSSYTFGQGTKLEIK

SEQ ID NO: 46 - protein, 4 aa, synthetic construct
  REGION 1..4: note = Linker
GGGS

SEQ ID NO: 47 - protein, 5 aa, synthetic construct
  REGION 1..5: note = Linker
GGGGS

SEQ ID NO: 48 - protein, 22 aa, synthetic construct
  REGION 1..22: note = GMCSFRa signal sequence
MLLLVTSLLLCELPHPAFLLIP